European Patent Specification EP 4 004 925 B1, published June 25, 2025. Title: Method for generating variants of a protein. Applicant: ECOLE POLYTECHNIQUE FEDERALE DE LAUSANNE (EPFL). The sequence listing filed with the application follows.

SEQUENCE LISTING (33 sequences)

SEQ ID NO: 1 - protein, 471 aa, Unknown
  Artificial sequences
MYPYDVPDYAYPYDVPDYAYPYDVPDYADDPLNLSWYDDDLERQNWSRPFNGSDGKADRPHYNYYATLLTLLIAVIVFGNVLVCMAVSREKALQTTTNYLIVSLAVADLLVATLVMPWVVYLEVVGEWKFSRIHCDIFVTLDVMMCTASILNLCAISIDRYTAVAMPMLYNTRYSSKRRVTVMISIVWVLSFTISCPLLFGLNNADQNECIIANPAFVVYSSIVSFYVPFIVTLLVYIKIYIVLRRRRKRVNTKRSSRAFRAHLRAPLKGNCTHPEDMKLCTVIMKSNGSFPVNRRRVEAARRAQELEMEMLSSTSPPERTRYSPIPPSHHQLTLPDPSHHGLHSTPDSPAKPEKNGHAKDHPKIAKIFEIQTMPNGKTRTSLKTMSRRKLSQQKEKKATQMLAIVLGVFIILWLPFFITHILNIHCDCNIPPVLYSAFTWLGYVNSAVNPIIYTTFNIEFRKAFLKILHC

SEQ ID NO: 2 - protein, 471 aa, Unknown
  Artificial sequence
MYPYDVPDYAYPYDVPDYAYPYDVPDYADDPLNLSWYDDDLERQNWSRPFNGSDGKADRPHYNYYATLLTLLIAVIVFGNVLVCMAVSREKALQTTTNYLIVSLAVADLLVATLVMPWVVYLEVVGEWKFSRIHCDIFVTLDVMMCTASILNLCAISIDRYTAVAMPMLYNTRYSSKRRVTVMISIVWVLSFTISCPLLFGLNNADQNECIIANPAFVVYSSIVSFYVPFIVTLLVYIKIYIVLRRRRKRVNTKRSSRAFRAHLRAPLKGNCTHPEDMKLCTVIMKSNGSFPVNRRRVEAARRAQELEMEMLSSTSPPERTRYSPIPPSHHQLTLPDPSHHGLHSTPDSPAKPEKNGHAKDHPKIAKIFEIQTMPNGKTRTSLKTMSRRKLSQQKEKKATQMLAIVLGVFIIVWLPFFITHILNIHCDCNIPPVLYSAFTWLGYVNSAVNPIIYTTFNIEFRKAFLKILHC

SEQ ID NO: 3 - protein, 471 aa, Unknown
  Artificial sequence
MYPYDVPDYAYPYDVPDYAYPYDVPDYADDPLNLSWYDDDLERQNWSRPFNGSDGKADRPHYNYYATLLTLLIAVIVFGNVLVCMAVSREKALQTTTNYLIVSLAVADLLVATLVMPWVVYLEVVGEWKFSRIHCDIFVTLDVMMCTASILNLCAISIDRYTAVAMPMLYNTRYSSKRRVTVMISIVWVLSFTISCPLLFGLNNADQNECIIANPAFVVYSSIVSFYVPMIVTLLVYIKIYIVLRRRRKRVNTKRSSRAFRAHLRAPLKGNCTHPEDMKLCTVIMKSNGSFPVNRRRVEAARRAQELEMEMLSSTSPPERTRYSPIPPSHHQLTLPDPSHHGLHSTPDSPAKPEKNGHAKDHPKIAKIFEIQTMPNGKTRTSLKTMSRRKLSQQKEKKATQMLAIVLGVFIICWLPFFITHILNIHCDCNIPPVLYSAFTWLGYVNSAVNPIIYTTFNIEFRKAFLKILHC

SEQ ID NO: 4 - protein, 471 aa, Unknown
  Artificial sequence
MYPYDVPDYAYPYDVPDYAYPYDVPDYADDPLNLSWYDDDLERQNWSRPFNGSDGKADRPHYNYYATLLTLLIAVIVFGNVLVCMAVSREKALQTTTNYLIVSLAVADLLVATLVMPWVVYLEVVGEWKFSRIHCDIFVTLDVMMCTASILNLCAISIDRYTAVAMPMLYNTRYSSKRRVTVMISIVWVLSFTISCPLLFGLNNADQNECIIANPAFVVYSSIVSFYVPFIVTLLVYIKIYIVLRRRRKRVNTKRSSRAFRAHLRAPLKGNCTHPEDMKLCTVIMKSNGSFPVNRRRVEAARRAQELEMEMLSSTSPPERTRYSPIPPSHHQLTLPDPSHHGLHSTPDSPAKPEKNGHAKDHPKIAKIFEIQTMPNGKTRTSLKTMSRRKLSQQKEKKATQMLAIVLGVIIILWLPFFITHILNIHCDCNIPPVLYSAFTWLGYVNSAVNPIIYTTFNIEFRKAFLKILHC

SEQ ID NO: 5 - protein, 471 aa, Unknown
  Artificial sequence
MYPYDVPDYAYPYDVPDYAYPYDVPDYADDPLNLSWYDDDLERQNWSRPFNGSDGKADRPHYNYYATLLTLLIAVIVFGNVLVCMAVSREKALQTTTNYLIVSLAVADLLVATLVMPWVVYLEVVGEWKFSRIHCDIFVTLDVMMCTASILNLCAISIDRYTAVAMPMLYNTRYSSKRRVTVMISIVWVLSFTISCPLLFGLNNADQNECIIANPAFVVYSSIVSFYVPFIVTLLVYIKIYIVLRRRRKRVNTKRSSRAFRAHLRAPLKGNCTHPEDMKLCTVIMKSNGSFPVNRRRVEAARRAQELEMEMLSSTSPPERTRYSPIPPSHHQLTLPDPSHHGLHSTPDSPAKPEKNGHAKDHPKIAKIFEIQTMPNGKTRTSLKTMSRRKLSQQKEKKATQMLAIVLGVIIICWLPFFITHILNIHCDCNIPPVLYSAFTWLGYVNSAVNPIIYTTFNIEFRKAFLKILHC

SEQ ID NO: 6 - protein, 471 aa, Unknown
  Artificial sequence
MYPYDVPDYAYPYDVPDYAYPYDVPDYADDPLNLSWYDDDLERQNWSRPFNGSDGKADRPHYNYYATLLTLLIAVIVFGNVLVCMAVSREKALQTTTNYLIVSLAVADLLVATLVMPWVVYLEVVGEWKFSRIHCDIFVTLDVMMCTASILNLCAISIDRYTAVAMPMLYNTRYSSKRRVTVMISIVWVLSFTISCPLLFGLNNADQNECIIANPAFVVYSSIVSFYVPFIVTLLVYIKIYIVLRRRRKRVNTKRSSRAFRAHLRAPLKGNCTHPEDMKLCTVIMKSNGSFPVNRRRVEAARRAQELEMEMLSSTSPPERTRYSPIPPSHHQLTLPDPSHHGLHSTPDSPAKPEKNGHAKDHPKIAKIFEIQTMPNGKTRTSLKTMSRRKLSQQKEKKATQMLAIVLGVYIICWLPFFITHILNIHCDCNIPPVLYSAFTWLGYVNSAVNPIIYTTFNIEFRKAFLKILHC

SEQ ID NO: 7 - protein, 471 aa, Unknown
  Artificial sequence
MYPYDVPDYAYPYDVPDYAYPYDVPDYADDPLNLSWYDDDLERQNWSRPFNGSDGKADRPHYNYYATLLTLLIAVIVFGNVLVCMAVSREKALQTTTNYLIVSLAVADLLVATLVMPWVVYLEVVGEWKFSRIHCDIFVTLDVMMCTASFLNLCAISIDRYTAVAMPMLYNTRYSSKRRVTVMISIVWVLSFTISCPLLFGLNNADQNECIIANPAFVVYSSIVSFYVPFIVTLLVYIKIYIVLRRRRKRVNTKRSSRAFRAHLRAPLKGNCTHPEDMKLCTVIMKSNGSFPVNRRRVEAARRAQELEMEMLSSTSPPERTRYSPIPPSHHQLTLPDPSHHGLHSTPDSPAKPEKNGHAKDHPKIAKIFEIQTMPNGKTRTSLKTMSRRKLSQQKEKKATQMLAIVLGVFIICWLPFFITHILNIHCDCNIPPVLYSAFTWLGYVNSAVNPIIYTTFNIEFRKAFLKILHC

SEQ ID NO: 8 - protein, 471 aa, Unknown
  Artificial sequence
MYPYDVPDYAYPYDVPDYAYPYDVPDYADDPLNLSWYDDDLERQNWSRPFNGSDGKADRPHYNYYATLLTLLIAVIVFGNVLVCMAVSREKALQTTTNYLIVSLAVADLLVATLVMPWVVYLEVVGEWKFSRIHCDIFVTLDVMMCTASLLNLCAISIDRYTAVAMPMLYNTRYSSKRRVTVMISIVWVLSFTISCPLLFGLNNADQNECIIANPAFVVYSSIVSFYVPFIVTLLVYIKIYIVLRRRRKRVNTKRSSRAFRAHLRAPLKGNCTHPEDMKLCTVIMKSNGSFPVNRRRVEAARRAQELEMEMLSSTSPPERTRYSPIPPSHHQLTLPDPSHHGLHSTPDSPAKPEKNGHAKDHPKIAKIFEIQTMPNGKTRTSLKTMSRRKLSQQKEKKATQMLAIVLGVFIICWLPFFITHILNIHCDCNIPPVLYSAFTWLGYVNSAVNPIIYTTFNIEFRKAFLKILHC

SEQ ID NO: 9 - protein, 471 aa, Unknown
  Artificial sequence
MYPYDVPDYAYPYDVPDYAYPYDVPDYADDPLNLSWYDDDLERQNWSRPFNGSDGKADRPHYNYYATLLTLLIAVIVFGNVLVCMAVSREKALQTTTNYLIVSLAVADLLVATLVMPWVVYLEVVGEWKFSRIHCDIFVTLDVMMCTASTLNLCAISIDRYTAVAMPMLYNTRYSSKRRVTVMISIVWVLSFTISCPLLFGLNNADQNECIIANPAFVVYSSIVSFYVPFIVTLLVYIKIYIVLRRRRKRVNTKRSSRAFRAHLRAPLKGNCTHPEDMKLCTVIMKSNGSFPVNRRRVEAARRAQELEMEMLSSTSPPERTRYSPIPPSHHQLTLPDPSHHGLHSTPDSPAKPEKNGHAKDHPKIAKIFEIQTMPNGKTRTSLKTMSRRKLSQQKEKKATQMLAIVLGVFIICWLPFFITHILNIHCDCNIPPVLYSAFTWLGYVNSAVNPIIYTTFNIEFRKAFLKILHC

SEQ ID NO: 10 - protein, 471 aa, Unknown
  Artificial sequence
MYPYDVPDYAYPYDVPDYAYPYDVPDYADDPLNLSWYDDDLERQNWSRPFNGSDGKADRPHYNYYATLLTLLIAVIVFGNVLVCMAVSREKALQTTTNYLIVSLAVADLLVATLVMPWVVYLEVVGEWKFSRIHCDIFVTLDVMMCTASILNLCAISIDRYTAVAMPMLYNTRYSSKRRVTVMISIVWVLSFTISCPLLFGLNNADQNECIIANPAFVVYSSIVSFYVPFIVTLLVYIKIYIVLRRRRKRVNTKRSSRAFRAHLRAPLKGNCTHPEDMKLCTVIMKSNGSFPVNRRRVEAARRAQELEMEMLSSTSPPERTRYSPIPPSHHQLTLPDPSHHGLHSTPDSPAKPEKNGHAKDHPKIAKIFEIQTMPNGKTRTSLKTMSRRKLSQQKEKKATQMLAIVIGVFIILWLPFFITHILNIHCDCNIPPVLYSAFTWLGYVNSAVNPIIYTTFNIEFRKAFLKILHC

SEQ ID NO: 11 - protein, 471 aa, Unknown
  Artificial sequence
MYPYDVPDYAYPYDVPDYAYPYDVPDYADDPLNLSWYDDDLERQNWSRPFNGSDGKADRPHYNYYATLLTLLIAVIVFGNVLVCMAVSREKALQTTTNYLIVSLAVADLLVATLVMPWVVYLEVVGEWKFSRIHCDIFVTLDVMMCTASILNLCAISIDRYTAVAMPMLYNTRYSSKRRVTVMISIVWVLSFTISCPLLFGLNNADQNECIIANPAFVVYSSIVSFYVPFIVTLLVYIKIYIVLRRRRKRVNTKRSSRAFRAHLRAPLKGNCTHPEDMKLCTVIMKSNGSFPVNRRRVEAARRAQELEMEMLSSTSPPERTRYSPIPPSHHQLTLPDPSHHGLHSTPDSPAKPEKNGHAKDHPKIAKIFEIQTMPNGKTRTSLKTMSRRKLSQQKEKKATQMLAIVIGVIIICWLPFFITHILNIHCDCNIPPVLYSAFTWLGYVNSAVNPIIYTTFNIEFRKAFLKILHC

SEQ ID NO: 12 - protein, 471 aa, Unknown
  Artificial sequence
MYPYDVPDYAYPYDVPDYAYPYDVPDYADDPLNLSWYDDDLERQNWSRPFNGSDGKADRPHYNYYATLLTLLIAVIVFGNVLVCMAVSREKALQTTTNYLIVSLAVADLLVATLVMPWVVYLEVVGEWKFSRIHCDIFVTLDVMMCTASILNLCAISIDRYTAVAMPMLYNTRYSSKRRVTVMISIVWVLSFTISCPLLFGLNNADQNECIIANPAFVVYSSIVSFYVPFIVTLLVYIKIYIVLRRRRKRVNTKRSSRAFRAHLRAPLKGNCTHPEDMKLCTVIMKSNGSFPVNRRRVEAARRAQELEMEMLSSTSPPERTRYSPIPPSHHQLTLPDPSHHGLHSTPDSPAKPEKNGHAKDHPKIAKIFEIQTMPNGKTRTSLKTMSRRKLSQQKEKKATQMLAIVIGVFIICWLPFFITHILNIHCDCNIPPVLYSAFTWLGYVNSAVNPIIYTTFNIEFRKAFLKILHC

SEQ ID NO: 13 - protein, 471 aa, Unknown
  Artificial sequence
MYPYDVPDYAYPYDVPDYAYPYDVPDYADDPLNLSWYDDDLERQNWSRPFNGSDGKADRPHYNYYATLLTLLIAVIVFGNVLVCMAVSREKALQTTTNYLIVSMAVADLLVATLVMPWVVYLEVVGEWKFSRIHCDIFVTLDVMMCTASILNLCAISIDRYTAVAMPMLYNTRYSSKRRVTVMISIVWVLSFTISCPLLFGLNNADQNECIIANPAFVVYSSIVSFYVPFIVTLLVYIKIYIVLRRRRKRVNTKRSSRAFRAHLRAPLKGNCTHPEDMKLCTVIMKSNGSFPVNRRRVEAARRAQELEMEMLSSTSPPERTRYSPIPPSHHQLTLPDPSHHGLHSTPDSPAKPEKNGHAKDHPKIAKIFEIQTMPNGKTRTSLKTMSRRKLSQQKEKKATQMLAIVLGVFIICWLPFFITHILNIHCDCNIPPVLYSAFTWLGYVNSAVNPIIYTTFNIEFRKAFLKILHC

SEQ ID NO: 14 - protein, 471 aa, Unknown
  Artificial sequence
MYPYDVPDYAYPYDVPDYAYPYDVPDYADDPLNLSWYDDDLERQNWSRPFNGSDGKADRPHYNYYATLLTLLIAVIVFGNVLVCMAVSREKALQTTTNYLIVSLAVADLLVATLVVPWVVYLEVVGEWKFSRIHCDIFVTLDVMMCTASILNLCAISIDRYTAVAMPMLYNTRYSSKRRVTVMISIVWVLSFTISCPLLFGLNNADQNECIIANPAFVVYSSIVSFYVPFIVTLLVYIKIYIVLRRRRKRVNTKRSSRAFRAHLRAPLKGNCTHPEDMKLCTVIMKSNGSFPVNRRRVEAARRAQELEMEMLSSTSPPERTRYSPIPPSHHQLTLPDPSHHGLHSTPDSPAKPEKNGHAKDHPKIAKIFEIQTMPNGKTRTSLKTMSRRKLSQQKEKKATQMLAIVLGVFIICWLPFFITHILNIHCDCNIPPVLYSAFTWLGYVNSAVNPIIYTTFNIEFRKAFLKILHC

SEQ ID NO: 15 - protein, 471 aa, Unknown
  Artificial sequence
MYPYDVPDYAYPYDVPDYAYPYDVPDYADDPLNLSWYDDDLERQNWSRPFNGSDGKADRPHYNYYATLLTLLIAVIVFGNVLVCMAVSREKALQTTTNYLIVSLAVADLLVATLVMPWVVYLEVVGEWKFSRIHCDIFVTLDVMMCTASILNLCAISIDRYTAVAMPMLYNTRYSSKRRVTVMISIVWVLSFTISCPLLFGLNNADQNECIIANPAFVVYSSIVSFYVPFIVTLLVYIKIYIVLRRRRKRVNTKRSSRAFRAHLRAPLKGNCTHPEDMKLCTVIMKSNGSFPVNRRRVEAARRAQELEMEMLSSTSPPERTRYSPIPPSHHQLTLPDPSHHGLHSTPDSPAKPEKNGHAKDHPKIAKIFEIQTMPNGKTRTSLKTMSRRKLSQQKEKKATQMLAIVLGVFIICWLPFFISHILNIHCDCNIPPVGYSAWTWLGYVNSAVNPIIYTTFNIEFRKAFLKILHC

SEQ ID NO: 16 - protein, 471 aa, Unknown
  Artificial sequence
MYPYDVPDYAYPYDVPDYAYPYDVPDYADDPLNLSWYDDDLERQNWSRPFNGSDGKADRPHYNYYATLLTLLIAVIVFGNVLVCMAVSREKALQTTTNYLYVSLAVADLLVATLVMPWVVYLEVVGEWKFSRIHCDIFVTLDVMMCTASILNLCAISIDRYTAVAMPMLYNTRYSSKRRVTVMISIVWVLSFTISCPLLFGLNNADQNECIIANPAFVVYSSIVSFYVPLIVIILVYIKIYIVLRRRRKRVNTKRSSRAFRAHLRAPLKGNCTHPEDMKLCTVIMKSNGSFPVNRRRVEAARRAQELEMEMLSSTSPPERTRYSPIPPSHHQLTLPDPSHHGLHSTPDSPAKPEKNGHAKDHPKIAKIFEIQTMPNGKTRTSLKTMSRRKLSQQKEKKATQLLAIYLGLFLICWLPFFISHILNIHCDCNIPPVGYSAWTWLGYVNSAINPIIFATFNIEFRKAFLKILHC

SEQ ID NO: 17 - protein, 471 aa, Unknown
  Artificial sequence
MYPYDVPDYAYPYDVPDYAYPYDVPDYADDPLNLSWYDDDLERQNWSRPFNGSDGKADRPHYNYYATLLTLLIAVIVFGNVLVCMAVSREKALQTTTNYLIVSLAVADLLVATLVMPWVVYLEVVGEWKFSRIHCDIFVTLDVMMCTASILNLCAISIDRYTAVAMPMLYNTRYSSKRRVTVMISIVWVLSFTISCPLLFGLNNADQNECIIANPAFVVYSSIVSFYVPLIVIILVYIKIYIVLRRRRKRVNTKRSSRAFRAHLRAPLKGNCTHPEDMKLCTVIMKSNGSFPVNRRRVEAARRAQELEMEMLSSTSPPERTRYSPIPPSHHQLTLPDPSHHGLHSTPDSPAKPEKNGHAKDHPKIAKIFEIQTMPNGKTRTSLKTMSRRKLSQQKEKKATQMLAIVLGVFLICWLPFFITHILNIHCDCNIPPVLYSAFTWLGYVNSAVNPIIYTTFNIEFRKAFLKILHC

SEQ ID NO: 18 - protein, 471 aa, Unknown
  Artificial sequence
MYPYDVPDYAYPYDVPDYAYPYDVPDYADDPLNLSWYDDDLERQNWSRPFNGSDGKADRPHYNYYATLLTLLIAVIVFGNVLVCMAVSREKALQTTTNYLIVSLAVADLLVATLVMPWVVYLEVVGEWKFSRIHCDIFVTLDVMMCTASILNLCAISIDRYTAVAMPMLYNTRYSSKRRVTVMISIVWVLSFTISCPLLFGLNNADQNECIIANPAFVVYSSIVSFYVPLIVIILVYIKIYIVLRRRRKRVNTKRSSRAFRAHLRAPLKGNCTHPEDMKLCTVIMKSNGSFPVNRRRVEAARRAQELEMEMLSSTSPPERTRYSPIPPSHHQLTLPDPSHHGLHSTPDSPAKPEKNGHAKDHPKIAKIFEIQTMPNGKTRTSLKTMSRRKLSQQKEKKATQLLAIYLGLFLICWLPFFITHILNIHCDCNIPPVLYSAFTWLGYVNSAINPIIYTTFNIEFRKAFLKILHC

SEQ ID NO: 19 - protein, 471 aa, Unknown
  Artificial sequence
MYPYDVPDYAYPYDVPDYAYPYDVPDYADDPLNLSWYDDDLERQNWSRPFNGSDGKADRPHYNYYATLLTLLIAVIVFGNVLVCMAVSREKALQTTTNYLYVSLAVADLLVATLVMPWVVYLEVVGEWKFSRIHCDIFVTLDVMMCTASILNLCAISIDRYTAVAMPMLYNTRYSSKRRVTVMISIVWVLSFTISCPLLFGLNNADQNECIIANPAFVVYSSIVSFYVPLIVIILVYIKIYIVLRRRRKRVNTKRSSRAFRAHLRAPLKGNCTHPEDMKLCTVIMKSNGSFPVNRRRVEAARRAQELEMEMLSSTSPPERTRYSPIPPSHHQLTLPDPSHHGLHSTPDSPAKPEKNGHAKDHPKIAKIFEIQTMPNGKTRTSLKTMSRRKLSQQKEKKATQLLAIYLGLFLICWLPFFITHILNIHCDCNIPPVLYSAFTWLGYVNSAINPIIFATFNIEFRKAFLKILHC

SEQ ID NO: 20 - protein, 471 aa, Unknown
  Artificial sequence
MYPYDVPDYAYPYDVPDYAYPYDVPDYADDPLNLSWYDDDLERQNWSRPFNGSDGKADRPHYNYYATLLTLLIAVIVFGNVLVCMAVSREKALQTTTNYLIVSLAVADLLVATLVMPWVVYLEVVGEWKFSRIHCDIFVTLDVMMCTASILNLCAISIDRYTAVAMPMLYNTRYSSKRRVTVMISIVWVLSFTISCPLLFGLNNADQNECIIANPAFVVYSSIVSFYVPFIVILLVYIKIYIVLRRRRKRVNTKRSSRAFRAHLRAPLKGNCTHPEDMKLCTVIMKSNGSFPVNRRRVEAARRAQELEMEMLSSTSPPERTRYSPIPPSHHQLTLPDPSHHGLHSTPDSPAKPEKNGHAKDHPKIAKIFEIQTMPNGKTRTSLKTMSRRKLSQQKEKKATQLLAIYLGLFIICWLPFFITHILNIHCDCNIPPVLYSAFTWLGYVNSAINPIIYTTFNIEFRKAFLKILHC

SEQ ID NO: 21 - protein, 471 aa, Unknown
  Artificial sequence
MYPYDVPDYAYPYDVPDYAYPYDVPDYADDPLNLSWYDDDLERQNWSRPFNGSDGKADRPHYNYYATLLTLLIAVIVFGNVLVCMAVSREKALQTTTNYLYVSLAVADLLVATLVMPWVVYLEVVGEWKFSRIHCDIFVTLDVMMCTASILNLCAISIDRYTAVAMPMLYNTRYSSKRRVTVMISIVWVLSFTISCPLLFGLNNADQNECIIANPAFVVYSSIVSFYVPFIVTLLVYIKIYIVLRRRRKRVNTKRSSRAFRAHLRAPLKGNCTHPEDMKLCTVIMKSNGSFPVNRRRVEAARRAQELEMEMLSSTSPPERTRYSPIPPSHHQLTLPDPSHHGLHSTPDSPAKPEKNGHAKDHPKIAKIFEIQTMPNGKTRTSLKTMSRRKLSQQKEKKATQMLAIVLGVFIICWLPFFITHILNIHCDCNIPPVLYSAFTWLGYVNSAVNPIIFATFNIEFRKAFLKILHC

SEQ ID NO: 22 - protein, 471 aa, Unknown
  Artificial sequence
MYPYDVPDYAYPYDVPDYAYPYDVPDYADDPLNLSWYDDDLERQNWSRPFNGSDGKADRPHYNYYATLLTLLIAVIVFGNVLVCMAVSREKALQTTTNYLIVSLAVADLLVATLVMPWVVYLEVVGEWKFSRIHCDIFVTLDVMMCTASILNLCAISIDRYTAVAMPMLYNTRYSSKRRVTVMISIVWVLSFTISCPLLFGLNNADQNECIIANPAFVVYSSIVSFYVPFIVILLVYIKIYIVLRRRRKRVNTKRSSRAFRAHLRAPLKGNCTHPEDMKLCTVIMKSNGSFPVNRRRVEAARRAQELEMEMLSSTSPPERTRYSPIPPSHHQLTLPDPSHHGLHSTPDSPAKPEKNGHAKDHPKIAKIFEIQTMPNGKTRTSLKTMSRRKLSQQKEKKATQMLAIVLGVFIICWLPFFITHILNIHCDCNIPPVLYSAFTWLGYVNSAVNPIIYTTFNIEFRKAFLKILHC

SEQ ID NO: 23 - protein, 471 aa, Unknown
  Artificial sequence
MYPYDVPDYAYPYDVPDYAYPYDVPDYADDPLNLSWYDDDLERQNWSRPFNGSDGKADRPHYNYYATLLTLLIAVIVFGNVLVCMAVSREKALQTTTNYLIVSLAVADLLVATLVMPWVVYLEVVGEWKFSRIHCDIFVTLDVMMCTASILNLCAISIDRYTAVAMPMLYNTRYSSKRRVTVMISIVWVLSFTISCPLLFGLNNADQNECIIANPAFVVYSSIVSFYVPFIVLLLVYIKIYIVLRRRRKRVNTKRSSRAFRAHLRAPLKGNCTHPEDMKLCTVIMKSNGSFPVNRRRVEAARRAQELEMEMLSSTSPPERTRYSPIPPSHHQLTLPDPSHHGLHSTPDSPAKPEKNGHAKDHPKIAKIFEIQTMPNGKTRTSLKTMSRRKLSQQKEKKATQMLAIVLGVFIICWLPFFITHILNIHCDCNIPPVLYSAFTWLGYVNSAVNPIIYTTFNIEFRKAFLKILHC

SEQ ID NO: 24 - protein, 471 aa, Unknown
  Artificial sequence
MYPYDVPDYAYPYDVPDYAYPYDVPDYADDPLNLSWYDDDLERQNWSRPFNGSDGKADRPHYNYYATLLTLLIAVIVFGNVLVCMAVSREKALQTTTNYLIVSLAVADLLVATLVMPWVVYLEVVGEWKFSRIHCDIFVTLDVMMCTASILNLCAISIDRYTAVAMPMLYNTRYSSKRRVTVMISIVWVLSFTISCPLLFGLNNADQNECIIANPAFVVYSSIVSFYVPFIVMLLVYIKIYIVLRRRRKRVNTKRSSRAFRAHLRAPLKGNCTHPEDMKLCTVIMKSNGSFPVNRRRVEAARRAQELEMEMLSSTSPPERTRYSPIPPSHHQLTLPDPSHHGLHSTPDSPAKPEKNGHAKDHPKIAKIFEIQTMPNGKTRTSLKTMSRRKLSQQKEKKATQMLAIVLGVFIILWLPFFITHILNIHCDCNIPPVLYSAFTWLGYVNSAVNPIIYTTFNIEFRKAFLKILHC

SEQ ID NO: 25 - protein, 471 aa, Unknown
  Artificial sequence
MYPYDVPDYAYPYDVPDYAYPYDVPDYADDPLNLSWYDDDLERQNWSRPFNGSDGKADRPHYNYYATLLTLLIAVIVFGNVLVCMAVSREKALQTTTNYLIVSLAVADLLVATLVMPWVVYLEVVGEWKFSRIHCDIFVTLDVMMCTASILNLCAISIDRYTAVAMPMLYNTRYSSKRRVTVMISIVWVLSFTISCPLLFGLNNADQNECIIANPAFVVYSSIVSFYVPFIVMLLVYIKIYIVLRRRRKRVNTKRSSRAFRAHLRAPLKGNCTHPEDMKLCTVIMKSNGSFPVNRRRVEAARRAQELEMEMLSSTSPPERTRYSPIPPSHHQLTLPDPSHHGLHSTPDSPAKPEKNGHAKDHPKIAKIFEIQTMPNGKTRTSLKTMSRRKLSQQKEKKATQMLAIVLGVFIIVWLPFFITHILNIHCDCNIPPVLYSAFTWLGYVNSAVNPIIYTTFNIEFRKAFLKILHC

SEQ ID NO: 26 - protein, 471 aa, Unknown
  Artificial sequence
MYPYDVPDYAYPYDVPDYAYPYDVPDYADDPLNLSWYDDDLERQNWSRPFNGSDGKADRPHYNYYATLLTLLIAVIVFGNVLVCMAVSREKALQTTTNYLIVSLAVADLLVATLVMPWVVYLEVVGEWKFSRIHCDIFVTLDVMMCTASILNLCAISIDRYTAVAMPMLYNTRYSSKRRVTVMISIVWVLSFTISCPLLFGLNNADQNECIIANPAFVVYSSIVSFYVPFIVMLLVYIKIYIVLRRRRKRVNTKRSSRAFRAHLRAPLKGNCTHPEDMKLCTVIMKSNGSFPVNRRRVEAARRAQELEMEMLSSTSPPERTRYSPIPPSHHQLTLPDPSHHGLHSTPDSPAKPEKNGHAKDHPKIAKIFEIQTMPNGKTRTSLKTMSRRKLSQQKEKKATQMLAIVLGVIIICWLPFFITHILNIHCDCNIPPVLYSAFTWLGYVNSAVNPIIYTTFNIEFRKAFLKILHC

SEQ ID NO: 27 - protein, 471 aa, Unknown
  Artificial sequence
MYPYDVPDYAYPYDVPDYAYPYDVPDYADDPLNLSWYDDDLERQNWSRPFNGSDGKADRPHYNYYATLLTLLIAVIVFGNVLVCMAVSREKALQTTTNYLIVSLAVADLLVATLVMPWVVYLEVVGEWKFSRIHCDIFVTLDVMMCTASILNLCAISIDRYTAVAMPMLYNTRYSSKRRVTVMISIVWVLSFTISCPLLFGLNNADQNECIIANPAFVVYSSIVSFYVPFIVMLLVYIKIYIVLRRRRKRVNTKRSSRAFRAHLRAPLKGNCTHPEDMKLCTVIMKSNGSFPVNRRRVEAARRAQELEMEMLSSTSPPERTRYSPIPPSHHQLTLPDPSHHGLHSTPDSPAKPEKNGHAKDHPKIAKIFEIQTMPNGKTRTSLKTMSRRKLSQQKEKKATQMLAIVIGVFIICWLPFFITHILNIHCDCNIPPVLYSAFTWLGYVNSAVNPIIYTTFNIEFRKAFLKILHC

SEQ ID NO: 28 - protein, 471 aa, Unknown
  Artificial sequence
MYPYDVPDYAYPYDVPDYAYPYDVPDYADDPLNLSWYDDDLERQNWSRPFNGSDGKADRPHYNYYATLLTLLIAVIVFGNVLVCMAVSREKALQTTTNYLIVSLAVADLLVATLVMPWVVYLEVVGEWKFSRIHCDIFVTLDVMMCTASILNLCAISIDRYTAVAMPMLYNTRYSSKRRVTVMISIVWVLSFTISCPLLFGLNNADQNECIIANPAFVVYSSIVSFYVPFIVVLLVYIKIYIVLRRRRKRVNTKRSSRAFRAHLRAPLKGNCTHPEDMKLCTVIMKSNGSFPVNRRRVEAARRAQELEMEMLSSTSPPERTRYSPIPPSHHQLTLPDPSHHGLHSTPDSPAKPEKNGHAKDHPKIAKIFEIQTMPNGKTRTSLKTMSRRKLSQQKEKKATQMLAIVLGVFIICWLPFFITHILNIHCDCNIPPVLYSAFTWLGYVNSAVNPIIYTTFNIEFRKAFLKILHC

SEQ ID NO: 29 - protein, 471 aa, Unknown
  Artificial sequence
MYPYDVPDYAYPYDVPDYAYPYDVPDYADDPLNLSWYDDDLERQNWSRPFNGSDGKADRPHYNYYATLLTLLIAVIVFGNVLVCMAVSREKALQTTTNYLIVSLAVADLLVATLVMPWVVYLEVVGEWKFSRIHCDIFVTLDVMMCTASILNLCAISIDRYTAVAMPMLYNTRYSSKRRVTVMISIVWVLSFTISCPLLFGLNNADQNECIIANPAFVVYSSIVSFYVPFIVTLLVLIKIYIVLRRRRKRVNTKRSSRAFRAHLRAPLKGNCTHPEDMKLCTVIMKSNGSFPVNRRRVEAARRAQELEMEMLSSTSPPERTRYSPIPPSHHQLTLPDPSHHGLHSTPDSPAKPEKNGHAKDHPKIAKIFEIQTMPNGKTRTSLKTMSRRKLSQQKEKKATQMLAIVLGVFIICWLPFFITHILNIHCDCNIPPVLYSAFTWLGYVNSAVNPIIYTTFNIEFRKAFLKILHC

SEQ ID NO: 30 - protein, 471 aa, Unknown
  Artificial sequence
MYPYDVPDYAYPYDVPDYAYPYDVPDYADDPLNLSWYDDDLERQNWSRPFNGSDGKADRPHYNYYATLLTLLIAVIVFGNVLVCMAVSREKALQTTTNYLIVSLAVADLLVATLVMPWVVYLEVVGEWKFSRIHCDIFVTLDVMMCTASILNLCAISIDRYTAVAMPMLYNTRYSSKRRVTVMISIVWVLSFTISCPLLFGLNNADQNECIIANPAFVVYSSIVSFYVPFIVTLLVYIKIYIVLRRRRKRVNTKRSSRAFRAHLRAPLKGNCTHPEDMKLCTVIMKSNGSFPVNRRRVEAARRAQELEMEMLSSTSPPERTRYSPIPPSHHQLTLPDPSHHGLHSTPDSPAKPEKNGHAKDHPKIAKIFEIQTMPNGKTRTSLKTMSRRKLSQQKEKKATQMLAIVLGVFIICWLPFFITHILNIHCDCNIPPVLYSAFTWLGYVNSAVNPIIFTTFNIEFRKAFLKILHC

SEQ ID NO: 31 - protein, 471 aa, Unknown
  Artificial sequence
MYPYDVPDYAYPYDVPDYAYPYDVPDYADDPLNLSWYDDDLERQNWSRPFNGSDGKADRPHYNYYATLLTLLIAVIVFGNVLVCMAVSREKALQTTTNYLIVSLAVADLLVATLVMPWVVYLEVVGEWKFSRIHCDIFVTLDVMMCTASILNLCAISIDRYTAVAMPMLYNTRYSSKRRVTVMISIVWVLSFTISCPLLFGLNNADQNECIIANPAFVVYSSIVSFYVPFIVMLLVYIKIYIVLRRRRKRVNTKRSSRAFRAHLRAPLKGNCTHPEDMKLCTVIMKSNGSFPVNRRRVEAARRAQELEMEMLSSTSPPERTRYSPIPPSHHQLTLPDPSHHGLHSTPDSPAKPEKNGHAKDHPKIAKIFEIQTMPNGKTRTSLKTMSRRKLSQQKEKKATQMLAIVLGVFIICWLPFFITHILNIHCDCNIPPVLYSAFTWLGYVNSAVNPIIYTTFNIEFRKAFLKILHC

SEQ ID NO: 32 - protein, 471 aa, Unknown
  Artificial sequence
MYPYDVPDYAYPYDVPDYAYPYDVPDYADDPLNLSWYDDDLERQNWSRPFNGSDGKADRPHYNYYATLLTLLIAVIVFGNVLVCMAVSREKALQTTTNYLIVSLAVADLLVATLVMPWVVYLEVVGEWKFSRIHCDIFVTLDVMMCTASILNLCAISIDRYTAVAMPMLYNTRYSSKRRVTVMISIVWVLSFTISCPLLFGLNNADQNECIIANPAFVVYSSIVSFYVPFIVTLLVYIKIYIVLRRRRKRVNTKRSSRAFRAHLRAPLKGNCTHPEDMKLCTVIMKSNGSFPVNRRRVEAARRAQELEMEMLSSTSPPERTRYSPIPPSHHQLTLPDPSHHGLHSTPDSPAKPEKNGHAKDHPKIAKIFEIQTMPNGKTRTSLKTMSRRKLSQQKEKKATQMLAIVLGVFIICWLPFFITHILNIHCDCNIPPVLYSAFTWLGYVNSAVNPIIYTTFNIEFRKAFLKILHC

SEQ ID NO: 33 - protein, 336 aa, Unknown
  Artificial sequence
MYPYDVPDYAYPYDVPDYAYPYDVPDYADDPLNLSWYDDDLERQNWSRPFNGSDGKADRPHYNYYATLLTLLIAVIVFGNVLVCMAVSREKALQTTTNYLIVSLAVADLLVATLVMPWVVYLEVVGEWKFSRIHCDIFVTLDVMMCTASILNLCAISIDRYTAVAMPMLYNTRYSSKRRVTVMISIVWVLSFTISCPLLFGLNNADQNECIIANPAFVVYSSIVSFYVPFIVTLLVYIKIYIVLRRRRKLVNTNRKLSQQKEKKATQLLAIYLGLFIICWLPFFITHILNIHCDCNPPVLYSAFTWLGYVNSAINPIIYTTFNIEFRKAFLKILHC